European Patent Application EP 4 814 118 A1, published September 30, 2026. Title: 一种VZV抗原变体、核酸、药物组合物及其应用. Applicant: 上海蓝鹊生物医药有限公司. The sequence listing filed with the application follows.

SEQUENCE LISTING (41 sequences)

SEQ ID NO: 1 - protein, 647 aa, synthetic construct
MGTVNKPVVGVLMGFGIITGTLRITNPVRASVLRYDDFHIDEDKLDTNSVYEPYYHSDHAESSWVNRGESSRKAYDHNSPYIWPRNDYDGFLENAHEHHGVYNQGRGIDSGERLMQPTQMSAQEDLGDDTGIHVIPTLNGDDRHKIVNVDQRQYGDVFKGDLNPKPQGQRLIEVSVEENHPFTLRAPIQRIYGVRYTETWSFLPSLTCTGDAAPAIQHICLKHTTCFQDVVVDVDCAENTKEDQLAEISYRFQGKKEADQPWIVVNTSTLFDELELDPPEIEPGVLKVLRTEKQYLGVYIWNMRGSDGTSTYATFLVTWKGDEKTRNPTPAVTPQPRGAEFHMWNYHSHVFSVGDTFSLAMHLQYKIHEAPFDLLLEWLYVPIDPTCQPMRLYSTCLYHPNAPQCLSHMNSGCTFTSPHLAQRVASTVYQNCEHADNYTAYCLGISHMEPSFGLILHDGGTTLKFVDTPESLSGLYVFVVYFNGHVEAVAYTVVSTVDHFVNAIEERGFPPTAGQPPATTKPKEITPVNPGTSPLLRYAAWTGGLAAVVLLCLVIFLICTAKRMRVKAYRVDKSPYNQSMYYAGLPVDDFEDSESTDTEEEFGNAIGGSHGGSSYTVYIDKTRYPYDVPDYAGSSGVSGWRLFKKIS

SEQ ID NO: 2 - protein, 647 aa, synthetic construct
MGTVNKPVVGVLMGFGIITGTLRITNPVRASVLRYDDFHIDEDKLDTNSVYEPYYHSDHAESSWVNRGESSRKAYDHNSPYIWPRNDYDGFLENAHEHHGVYNQGRGIDSGERLMQPTQMSAQEDLGDDTGIHVIPTLNGDDRHKIVNVDQRQYGDVFKGDLNPKPQGQRLIEVSVEENHPFTLRAPIQRIYGVRYTETWSFLPSLTCTGDAAPAIQHICLKHTTCFQDVVVDVDCAENTKEDQLAEISYRFQGKKEADQPWIVVNTSTLFDELELDPPEIEPGVLKVLRTEKQYLGVYIWNMRGSDGTSTYATFLVTWKGDEKTRNPTPAVTPQPRGAEFHMWNYHSHVFSVGDTFSLAMHLQYKIHEAPFDLLLEWLYVPIDPTCQPMRLYSTCLYHPNAPQCLSHMNSGCTFTSPHLAQRVASTVYQNCEHADNYTAYCLGISHMEPSFGLILHDGGTTLKFVDTPESLSGLYVFVVYFNGHVEAVAYTVVSTVDHFVNAIEERGFPPTAGQPPATTKPKEITPVNPGTSPLLRYAAWTGGLAAVVLLCLVIFLICTAKRMRVKAARVDKSPYNQSMYYAGLPVDDFEDAEAADAEEEFGNAIGGSHGGSSYTVYIDKTRYPYDVPDYAGSSGVSGWRLFKKIS

SEQ ID NO: 3 - protein, 584 aa, synthetic construct
MGTVNKPVVGVLMGFGIITGTLRITNPVRASVLRYDDFHIDEDKLDTNSVYEPYYHSDHAESSWVNRGESSRKAYDHNSPYIWPRNDYDGFLENAHEHHGVYNQGRGIDSGERLMQPTQMSAQEDLGDDTGIHVIPTLNGDDRHKIVNVDQRQYGDVFKGDLNPKPQGQRLIEVSVEENHPFTLRAPIQRIYGVRYTETWSFLPSLTCTGDAAPAIQHICLKHTTCFQDVVVDVDCAENTKEDQLAEISYRFQGKKEADQPWIVVNTSTLFDELELDPPEIEPGVLKVLRTEKQYLGVYIWNMRGSDGTSTYATFLVTWKGDEKTRNPTPAVTPQPRGAEFHMWNYHSHVFSVGDTFSLAMHLQYKIHEAPFDLLLEWLYVPIDPTCQPMRLYSTCLYHPNAPQCLSHMNSGCTFTSPHLAQRVASTVYQNCEHADNYTAYCLGISHMEPSFGLILHDGGTTLKFVDTPESLSGLYVFVVYFNGHVEAVAYTVVSTVDHFVNAIEERGFPPTAGQPPATTKPKEITPVNPGTSPLLRYAAWTGGLAAVVLLCLVIFLICTYPYDVPDYAGSSGVSGWRLFKKIS

SEQ ID NO: 4 - protein, 597 aa, synthetic construct
MGTVNKPVVGVLMGFGIITGTLRITNPVRASVLRYDDFHIDEDKLDTNSVYEPYYHSDHAESSWVNRGESSRKAYDHNSPYIWPRNDYDGFLENAHEHHGVYNQGRGIDSGERLMQPTQMSAQEDLGDDTGIHVIPTLNGDDRHKIVNVDQRQYGDVFKGDLNPKPQGQRLIEVSVEENHPFTLRAPIQRIYGVRYTETWSFLPSLTCTGDAAPAIQHICLKHTTCFQDVVVDVDCAENTKEDQLAEISYRFQGKKEADQPWIVVNTSTLFDELELDPPEIEPGVLKVLRTEKQYLGVYIWNMRGSDGTSTYATFLVTWKGDEKTRNPTPAVTPQPRGAEFHMWNYHSHVFSVGDTFSLAMHLQYKIHEAPFDLLLEWLYVPIDPTCQPMRLYSTCLYHPNAPQCLSHMNSGCTFTSPHLAQRVASTVYQNCEHADNYTAYCLGISHMEPSFGLILHDGGTTLKFVDTPESLSGLYVFVVYFNGHVEAVAYTVVSTVDHFVNAIEERGFPPTAGQPPATTKPKEITPVNPGTSPLLRYAAWTGGLAAVVLLCLVIFLICTAKRMRVKAARVDKYPYDVPDYAGSSGVSGWRLFKKIS

SEQ ID NO: 5 - protein, 647 aa, synthetic construct
MGTVNKPVVGVLMGFGIITGTLRITNPVRASVLRYDDFHIDEDKLDTNSVYEPYYHSDHAESSWVNRGESSRKAYDHNSPYIWPRNDYDGFLENAHEHHGVYNQGRGIDSGERLMQPTQMSAQEDLGDDTGIHVIPTLNGDDRHKIVNVDQRQYGDVFKGDLNPKPQGQRLIEVSVEENHPFTLRAPIQRIYGVRYTETWSFLPSLTCTGDAAPAIQHICLKHTTCFQDVVVDVDCAENTKEDQLAEISYRFQGKKEADQPWIVVNTSTLFDELELDPPEIEPGVLKVLRTEKQYLGVYIWNMRGSDGTSTYATFLVTWKGDEKTRNPTPAVTPQPRGAEFHMWNYHSHVFSVGDTFSLAMHLQYKIHEAPFDLLLEWLYVPIDPTCQPMRLYSTCLYHPNAPQCLSHMNSGCTFTSPHLAQRVASTVYQNCEHADNYTAYCLGISHMEPSFGLILHDGGTTLKFVDTPESLSGLYVFVVYFNGHVEAVAYTVVSTVDHFVNAIEERGFPPTAGQPPATTKPKEITPVNPGTSPLLRYAAWTGGLAAVVLLCLVIFLICTAKRMRVKAARVDKSPYNQSMYGAGLPVDDFEDAEAADAEEEFGNAIGGSHGGSSYTVYIDKTRYPYDVPDYAGSSGVSGWRLFKKIS

SEQ ID NO: 6 - protein, 592 aa, synthetic construct
MGTVNKPVVGVLMGFGIITGTLRITNPVRASVLRYDDFHIDEDKLDTNSVYEPYYHSDHAESSWVNRGESSRKAYDHNSPYIWPRNDYDGFLENAHEHHGVYNQGRGIDSGERLMQPTQMSAQEDLGDDTGIHVIPTLNGDDRHKIVNVDQRQYGDVFKGDLNPKPQGQRLIEVSVEENHPFTLRAPIQRIYGVRYTETWSFLPSLTCTGDAAPAIQHICLKHTTCFQDVVVDVDCAENTKEDQLAEISYRFQGKKEADQPWIVVNTSTLFDELELDPPEIEPGVLKVLRTEKQYLGVYIWNMRGSDGTSTYATFLVTWKGDEKTRNPTPAVTPQPRGAEFHMWNYHSHVFSVGDTFSLAMHLQYKIHEAPFDLLLEWLYVPIDPTCQPMRLYSTCLYHPNAPQCLSHMNSGCTFTSPHLAQRVASTVYQNCEHADNYTAYCLGISHMEPSFGLILHDGGTTLKFVDTPESLSGLYVFVVYFNGHVEAVAYTVVSTVDHFVNAIEERGFPPTAGQPPATTKPKEITPVNPGTSPLLRYAAWTGGLAAVVLLCLVIFLICTAKRMRVKAYPYDVPDYAGSSGVSGWRLFKKIS

SEQ ID NO: 7 - protein, 575 aa, synthetic construct
MGTVNKPVVGVLMGFGIITGTLRITNPVRASVLRYDDFHIDEDKLDTNSVYEPYYHSDHAESSWVNRGESSRKAYDHNSPYIWPRNDYDGFLENAHEHHGVYNQGRGIDSGERLMQPTQMSAQEDLGDDTGIHVIPTLNGDDRHKIVNVDQRQYGDVFKGDLNPKPQGQRLIEVSVEENHPFTLRAPIQRIYGVRYTETWSFLPSLTCTGDAAPAIQHICLKHTTCFQDVVVDVDCAENTKEDQLAEISYRFQGKKEADQPWIVVNTSTLFDELELDPPEIEPGVLKVLRTEKQYLGVYIWNMRGSDGTSTYATFLVTWKGDEKTRNPTPAVTPQPRGAEFHMWNYHSHVFSVGDTFSLAMHLQYKIHEAPFDLLLEWLYVPIDPTCQPMRLYSTCLYHPNAPQCLSHMNSGCTFTSPHLAQRVASTVYQNCEHADNYTAYCLGISHMEPSFGLILHDGGTTLKFVDTPESLSGLYVFVVYFNGHVEAVAYTVVSTVDHFVNAIEERGFPPTAGQPPATTKPKEITPVNPGTSPLLRQILAIYSTVASSLVLVVSLGAISFWMCSNGSLQCRICI

SEQ ID NO: 8 - protein, 581 aa, synthetic construct
MGTVNKPVVGVLMGFGIITGTLRITNPVRASVLRYDDFHIDEDKLDTNSVYEPYYHSDHAESSWVNRGESSRKAYDHNSPYIWPRNDYDGFLENAHEHHGVYNQGRGIDSGERLMQPTQMSAQEDLGDDTGIHVIPTLNGDDRHKIVNVDQRQYGDVFKGDLNPKPQGQRLIEVSVEENHPFTLRAPIQRIYGVRYTETWSFLPSLTCTGDAAPAIQHICLKHTTCFQDVVVDVDCAENTKEDQLAEISYRFQGKKEADQPWIVVNTSTLFDELELDPPEIEPGVLKVLRTEKQYLGVYIWNMRGSDGTSTYATFLVTWKGDEKTRNPTPAVTPQPRGAEFHMWNYHSHVFSVGDTFSLAMHLQYKIHEAPFDLLLEWLYVPIDPTCQPMRLYSTCLYHPNAPQCLSHMNSGCTFTSPHLAQRVASTVYQNCEHADNYTAYCLGISHMEPSFGLILHDGGTTLKFVDTPESLSGLYVFVVYFNGHVEAVAYTVVSTVDHFVNAIEERGFPPTAGQPPATTKPKEITPVNPGTSPLLRWPWYIWLGFIAGLIAIVMVTIMLCCMTSCCSCLKGCCSCGSCCK

SEQ ID NO: 9 - protein, 623 aa, synthetic construct
MGTVNKPVVGVLMGFGIITGTLRITNPVRASVLRYDDFHIDEDKLDTNSVYEPYYHSDHAESSWVNRGESSRKAYDHNSPYIWPRNDYDGFLENAHEHHGVYNQGRGIDSGERLMQPTQMSAQEDLGDDTGIHVIPTLNGDDRHKIVNVDQRQYGDVFKGDLNPKPQGQRLIEVSVEENHPFTLRAPIQRIYGVRYTETWSFLPSLTCTGDAAPAIQHICLKHTTCFQDVVVDVDCAENTKEDQLAEISYRFQGKKEADQPWIVVNTSTLFDELELDPPEIEPGVLKVLRTEKQYLGVYIWNMRGSDGTSTYATFLVTWKGDEKTRNPTPAVTPQPRGAEFHMWNYHSHVFSVGDTFSLAMHLQYKIHEAPFDLLLEWLYVPIDPTCQPMRLYSTCLYHPNAPQCLSHMNSGCTFTSPHLAQRVASTVYQNCEHADNYTAYCLGISHMEPSFGLILHDGGTTLKFVDTPESLSGLYVFVVYFNGHVEAVAYTVVSTVDHFVNAIEERGFPPTAGQPPATTKPKEITPVNPGTSPLLRYAAWTGGLAAVVLLCLVIFLICTAKRMRVKAARVDKSPYNQSMYGAGLPVDDFEDAEAADAEEEFGNAIGGSHGGSSYTVYIDKTR

SEQ ID NO: 10 - protein, 44 aa, synthetic construct
WPWYIWLGFIAGLIAIVMVTIMLCCMTSCCSCLKGCCSCGSCCK

SEQ ID NO: 11 - protein, 38 aa, synthetic construct
QILAIYSTVASSLVLVVSLGAISFWMCSNGSLQCRICI

SEQ ID NO: 12 - RNA, 1941 nt, synthetic construct
  source 1..1941: mol_type = other RNA
atgggcaccgtgaataagccagtggtgggcgtgctgatgggctttggcattatcaccggaacactgaggatcaccaacccagtgagggcctctgtgctgagatacgacgacttccacatcgacgaggacaagctggacaccaacagcgtgtacgagccatactaccacagcgatcatgccgagagctcttgggtgaacaggggagagagcagcaggaaggcctacgaccacaattctccctatatctggcccaggaacgactacgatggcttcctggagaatgcccatgaacaccacggagtgtacaaccagggcagaggcattgactctggagagaggctgatgcagccaacccagatgtctgcccaggaggatctgggagacgataccggcatccatgtgattcccacactgaacggagacgacaggcacaagatcgtgaatgtggaccagagacagtacggcgatgtgttcaagggcgacctgaatcctaagcctcagggccagcgactgattgaggtgtctgtggaggagaaccatcctttcacactgcgggctcctatccagcggatctacggcgtgagatacaccgaaacctggagctttctgccaagcctgacctgtacaggcgatgccgctcctgctatccagcacatctgcctgaagcatacaacatgctttcaggacgtggtggtggatgtggattgcgccgagaacaccaaagaggaccagctggccgagattagctacagattccagggcaagaaggaggccgatcagccctggatcgtggtgaatacctctaccctgtttgacgagctggagctggacccccctgagattgagcctggagtgctgaaggtgctgagaacagagaagcagtacctgggcgtgtacatttggaacatgagaggcagcgacggcacctctacctatgccacatttctggtgacctggaagggcgacgagaaaaccagaaatccaacacctgccgtgacaccccagcccaggggagccgagtttcacatgtggaattaccacagccacgtgttcagcgtgggcgacacatttagcctggccatgcacctgcagtacaaaatccacgaggctcctttcgatctgctgctggagtggctgtatgtgcctattgaccctacctgccagcctatgaggctgtacagcacctgtctgtaccacccaaacgcccctcagtgcctgagccatatgaacagcggctgtacattcacctctccacacctggcccagagagtggccagcaccgtgtatcagaattgcgagcatgccgataactacacagcctactgtctgggcattagccacatggagcctagctttggcctgatcctgcacgatggaggcaccaccctgaaattcgtggatacccccgagagcctgagcggcctgtacgtgtttgtggtgtacttcaatggacacgtggaggccgtggcctacacagtggtgagcacagtggatcacttcgtgaacgctattgaggagagaggatttcctccaacagccggccagcctccagccacaaccaaacccaaagaaatcacccccgtgaatcctggaacatctcccctgctgaggtatgctgcttggacaggaggcctggctgccgtggtgctgctgtgcctggtgatctttctgatctgtaccgctaagagaatgagggtgaaggcctatagagtggacaagagcccctacaaccagagcatgtactacgccggcctgcctgtggacgattttgaggatagcgagagcacagataccgaggaggagtttggcaatgccatcggcggcagccatggcggcagcagctacaccgtgtacatcgataagaccaggtatccatacgatgtgcccgattatgccggatcttctggagtgtctggctggcggctgttcaagaagatcagc

SEQ ID NO: 13 - RNA, 1941 nt, synthetic construct
  source 1..1941: mol_type = other RNA
atgggcaccgtgaacaagcctgtggtgggagtgctgatgggcttcggaatcattacaggcacactgagaatcaccaatcctgtgagagccagcgtgctgcggtacgacgacttccacatcgacgaggacaagctggacaccaacagcgtgtacgagccctactaccacagcgaccacgccgagagcagctgggtgaataggggcgaatctagcagaaaagcctacgaccacaatagcccttacatctggcctaggaacgattacgacggatttctggagaatgctcacgagcaccacggcgtgtacaatcagggcaggggcattgactctggcgagaggctgatgcagcctacccagatgagcgcccaggaagatctgggcgacgacacaggcatccatgtgatccctacactgaatggagacgacagacacaagatcgtgaatgtggatcagagacagtacggcgacgtgtttaaaggcgatctgaaccccaagcctcagggccagcggctgatcgaggtgtctgtggaggagaaccacccttttacactgcgggcccctatccagcggatctacggcgtgagatacacagagacatggagcttcctgccttctctgacctgtacaggagacgctgctcctgccattcagcacatctgcctgaaacacaccacatgctttcaggacgtggtggtggacgtggattgtgccgagaataccaaggaggaccagctggccgagatcagctacaggttccagggaaagaaggaggccgaccagccttggattgtggtgaacacctctaccctgtttgatgagctggagctggaccctccagagattgagcccggcgtgctgaaagtgctgagaaccgagaagcagtatctgggcgtgtatatctggaacatgaggggcagcgatggaaccagcacctacgccaccttcctggtgacatggaagggcgacgagaagacaaggaatcctacaccagccgtgacacctcagccaagaggcgccgagtttcacatgtggaattatcactctcacgtgttcagcgtgggcgacaccttcagcctggccatgcatctgcagtataagatccacgaggccccctttgatctgctgctggagtggctgtatgtgcctatcgacccaacctgccagccaatgaggctgtactctacctgcctgtaccacccaaacgcccctcagtgcctgagccacatgaacagcggctgtacatttacaagcccccatcttgctcagagggtggcctctacagtgtaccagaattgcgagcacgccgataattacacagcctactgcctgggcatcagccacatggagcctagctttggcctgatcctgcacgatggcggcaccaccctgaagtttgtggatacacctgagagcctgagcggcctgtacgtgttcgtggtgtactttaacggacatgtggaggccgtggcctatacagtggtgagcaccgtggaccattttgtgaatgccattgaggagagaggattccctcctacagccggacagcctccagccaccaccaagccaaaggaaatcacacccgtgaatccaggaacctctcctctgctgagatatgctgcctggacaggcggcctggctgctgtggtgctgctgtgtctggttatcttcctgatctgtacagctaagaggatgcgggtgaaggcctacagggtggataagagcccatacaaccagagcatgtactacgccggcctgcctgtggatgatttcgaggatagcgaaagcaccgataccgaggaggagtttggcaacgccattggcggctctcacggcggcagcagctacaccgtgtatattgacaagaccaggtacccttacgatgtgccagattacgccggaagctctggcgtgtctggctggcggctgttcaagaagatcagc

SEQ ID NO: 14 - RNA, 1941 nt, synthetic construct
  source 1..1941: mol_type = other RNA
atgggcaccgtgaataagcccgtggtgggcgtgctgatgggctttggcatcatcacaggaacactgagaatcaccaaccctgtgagagccagcgtgctgagatacgacgactttcacatcgacgaggacaagctggacaccaacagcgtgtacgagccttactaccacagcgaccacgccgagagcagctgggtgaataggggagagagcagcaggaaggcctacgaccacaatagcccatacatctggcccagaaacgattacgatggctttctggaaaacgcccacgagcatcacggagtgtacaatcagggaaggggcattgatagcggcgaaaggctgatgcagcccacccagatgtctgcccaggaggatctgggagatgataccggcattcacgtgatccccaccctgaatggcgacgacaggcacaagatcgtgaacgtggaccagagacagtatggcgacgtgttcaaaggagatctgaaccctaagcctcagggacagaggctgattgaggtgagcgtggaggagaaccacccttttaccctgcgggcccctatccagagaatctacggcgtgagatacaccgaaacatggagcttcctgccttctctgacatgcacaggcgatgccgcccctgccatccagcacatctgcctgaagcacacaacatgctttcaggatgtggtggtggatgtggattgtgccgagaacacaaaggaggaccagctggccgagatctcttacagattccagggcaagaaggaggccgaccagccttggatcgtggtgaatacctctaccctgttcgatgagctggagctggacccaccagagatcgagcctggcgtgctcaaggtgctgagaaccgagaaacagtacctgggcgtgtacatttggaacatgagaggctctgacggcacatctacctacgccacctttctggtgacctggaagggagacgagaagaccagaaacccaacacctgccgtgacaccccagccaagaggcgccgagtttcacatgtggaattatcacagccacgtgttcagcgtgggcgacaccttcagcctggctatgcatctgcagtataagatccacgaagccccattcgacctgctgctggagtggctgtatgtgccaatcgacccaacatgccagcccatgcgcctgtacagcacctgtctgtatcatcctaacgccccacagtgcttaagccacatgaacagcggctgtacattcacatctccacacctcgcccagagggtggccagcaccgtgtaccagaattgtgaacatgccgacaattacaccgcctactgcctgggaatcagccacatggagcctagcttcggcctgatcctgcacgatggaggcacaaccctgaagtttgtggacacacccgagtcactgagcggcctgtacgtgtttgtggtgtacttcaatggacacgtggaggccgtggcctacacagtggtgtctaccgtggatcatttcgtgaacgctatcgaggagagaggatttcctcctacagctggacagcctcccgccaccaccaaacccaaggagattacacctgtgaatccaggcacatctcccctgctgcggtatgctgcttggacaggaggcctggctgctgtggtgctgctgtgtctggtgatcttcctgatctgcaccgctaaaagaatgagggtgaaagcctaccgggtggataaaagcccttacaaccagagcatgtactacgccggcctgcccgtggatgactttgaagacagcgagagcaccgataccgaagaggagtttggcaatgccatcggcggctcccacggcggcagcagctataccgtgtacatcgacaagaccagatacccttacgatgtccctgactatgccggctctagcggagtgtctggctggagattgttcaagaagatcagc

SEQ ID NO: 15 - RNA, 1941 nt, synthetic construct
  source 1..1941: mol_type = other RNA
atgggcaccgtgaacaagcctgtggtgggcgtgctgatgggatttggaatcatcaccggcaccctgagaatcaccaaccctgtgagagccagcgtgctgaggtatgacgacttccatatcgacgaggacaagctggacaccaatagcgtgtacgagccctactaccacagcgaccacgccgagagctcttgggtgaatagaggagagagcagcaggaaggcctacgatcacaacagcccttacatctggcccagaaacgactatgacggcttcctggaaaacgcccacgagcaccatggcgtgtataatcagggcagaggaatcgatagcggagagaggctgatgcaacctacccagatgtctgcccaggaggatctgggcgatgataccggaatccacgtgatccctaccctgaacggcgacgacagacacaagatcgtgaatgtggaccagagacagtacggcgatgtgttcaagggcgatctgaaccccaaacctcagggacagaggctcatcgaggtgagcgtggaggagaaccatccttttaccctgagggcccctatccagagaatctacggcgtgaggtataccgagacatggtccttcctgcccagcctgacctgtacaggcgatgccgctcctgccatccagcatatttgcctgaagcataccacctgttttcaggatgtggtggtggatgtggattgcgccgagaacaccaaggaggaccagctggccgagatctcttatagattccagggcaagaaggaggccgaccagccttggattgtggtgaacacctctaccctgttcgacgagctggagctggacccccctgagattgaaccaggcgttctgaaggtgctgagaaccgagaagcagtacctgggagtgtacatctggaatatgagaggcagcgatggcaccagcacctacgctacctttctggtgacctggaagggagacgagaaaaccaggaatccaacccctgccgtgacaccacagcccagaggcgccgagtttcacatgtggaattaccacagccacgtgttcagcgtgggcgacaccttctctctggccatgcacctgcagtataagattcacgaagctccatttgacctgctgctggagtggctgtacgtgccaattgaccccacatgccagccaatgaggctgtacagcacctgcctgtaccatccaaacgccccccagtgcctgtctcacatgaacagcggctgtacatttacaagccctcacctggcccagcgagtggccagcacagtgtaccagaattgtgagcatgctgacaattacacagcctattgcctgggcatcagccacatggagccatctttcggcctgatcctgcacgatggcggcaccaccctgaaatttgtggatacccctgagagcctgagcggcctgtacgtgtttgtggtgtactttaacggccacgtggaggccgtggcctacaccgtggtgagcacagtggatcattttgtgaatgccatcgaagaaagaggcttccctcctacagccggacagcctcctgccacaacaaagcccaaggagattaccccagtgaatccaggaacctctccactgctgagatacgccgcttggacaggaggcctggctgctgtggtgctgctgtgcctggtgatcttcctgatttgcaccgctaagagaatgagagtgaaagccgccagagtggataagagcccctacaaccagagcatgtactatgccggcctgcctgtggatgatttcgaagatgccgaagctgccgatgctgaggaggagtttggcaatgccattggcggcagccacggcggcagcagctataccgtgtacatcgacaagacaaggtacccttacgacgtgcccgattatgctggaagctctggagtgtctggctggaggctgttcaagaagatcagc

SEQ ID NO: 16 - RNA, 1941 nt, synthetic construct
  source 1..1941: mol_type = other RNA
atgggcaccgtgaacaagcctgtggtgggcgtgctcatgggctttggcatcatcacaggcaccctgagaatcaccaatcccgtgagagccagcgtgctgcggtacgacgacttccacatcgacgaggacaagctggacaccaatagcgtgtacgagccctactaccacagcgaccacgccgagagcagctgggtgaatagaggagaatctagcaggaaggcctatgaccacaatagcccatacatttggcccaggaatgattacgacggcttcctggagaacgcccacgagcaccacggcgtgtacaaccagggaagaggcattgattctggcgaacggctgatgcagccaacacagatgagcgcccaggaggacctgggagatgataccggaatccacgtgattcctaccctgaacggcgatgatagacacaagatcgtgaacgtggaccagagacagtacggcgacgtgtttaagggcgacctgaaccccaagcctcagggacagaggctgattgaggtgagcgtggaagagaaccaccctttcacactgagagcccccatccagaggatttacggcgtgaggtacacagagacatggagctttctgcctagcctgacatgtacaggcgatgccgcccctgccattcagcacatctgcctgaagcacaccacctgttttcaggatgtggtggtggatgtggattgcgccgagaacaccaaggaggatcagctggccgagatcagctacagattccagggaaagaaggaggccgaccagccttggatcgtggtgaatacaagcaccctgttcgatgagctggagctggaccctcccgagattgaacctggcgtgctgaaggtgctgaggaccgagaagcagtatctgggagtgtacatttggaatatgaggggcagcgacggcacatctacctacgccaccttcctggtgacatggaagggcgacgaaaaaacccggaatcctacccctgccgtgaccccacagcctagaggagccgagtttcacatgtggaattaccacagccacgtgttcagcgtgggagacacattctctctggccatgcacctgcagtacaagattcacgaagccccattcgacctgctgctggagtggctgtatgtgcccattgatcccacctgtcagcccatgcgactgtacagcacctgtctgtatcacccaaacgccccccagtgtctgtctcacatgaatagcggatgcacctttacaagcccacatctggcccagagggtggctagcacagtgtaccagaattgcgagcacgccgacaactacacagcttactgcctgggcatcagccacatggagccttctttcggcctgatcctgcacgacggcggcacaacactgaaatttgtggataccccagagagcctgtctggcctgtacgtgtttgtggtgtattttaacggccacgtggaggccgtggcctacacagtggtgtctaccgtggaccactttgtgaacgctatcgaggagagaggctttcctccaacagctggacagcctccagctaccacaaagcctaaggagatcacccctgtgaaccccggaacatctccactgctgagatacgccgcttggaccggcggattggctgccgttgtgctgctgtgcctggtgatctttctgatttgtacagccaagagaatgagagtgaaggctgctcgggtggacaagagcccttacaatcagagcatgtactacgccggcctgcctgtggatgacttcgaagatgccgaagctgccgatgccgaggaggaatttggcaatgctatcggcggcagccatggcggcagcagctacaccgtgtacatcgacaaaaccaggtatccatacgatgtgcccgattatgccggatcttctggcgtgagcggctggagattgttcaagaagatctcc

SEQ ID NO: 17 - RNA, 1941 nt, synthetic construct
  source 1..1941: mol_type = other RNA
atgggcaccgtgaacaagcctgtggtgggagtgctcatgggatttggaatcattacaggcacactgaggatcaccaaccccgtgagagccagcgtgctgaggtacgatgacttccacatcgacgaggacaagctggacaccaacagcgtgtacgagccctactaccacagcgaccacgccgagagctcttgggtgaataggggcgaatctagcagaaaggcctacgaccacaatagcccctatatttggcctagaaacgactacgatggcttcctggagaacgcccacgagcaccacggagtgtacaatcagggcagaggcatcgatagcggcgaaaggctgatgcagcctacccagatgagcgcccaggaagatctgggcgatgacacaggcatccatgtgattcctacactgaacggcgacgacaggcacaaaatcgtgaatgtggatcagaggcagtacggcgacgtgtttaagggcgatctgaatcccaagccacagggccagaggctgatcgaagtgagcgtggaggagaatcacccttttaccctgcgggccccaatccagcggatctacggagtgaggtataccgaaacatggagctttctgccaagcctgacctgtaccggagacgctgcccctgctatccagcacatttgtctgaagcacaccacctgttttcaggacgtggtggtggatgtggattgtgccgagaacaccaaggaggaccagctggccgagatcagctacagattccagggcaagaaggaggccgatcagccatggattgttgtgaataccagcaccctgttcgacgagctggagctggaccctccagaaattgagcctggcgtgctgaaggtgctgagaaccgagaaacagtacctgggagtttacatctggaacatgaggggctccgacggcacaagcacctacgctaccttcctggtgacatggaagggcgacgagaagacaagaaatcctaccccagccgtgacaccacagcccaggggcgccgagtttcatatgtggaattaccacagccacgtgttcagcgtgggcgatacatttagcctggccatgcatctgcagtacaagatccacgaggctcctttcgacctgctgctggaatggctgtacgtgccaatcgaccccacatgccagcctatgaggctgtatagcacatgcctgtatcaccctaacgccccccagtgcctgagccacatgaacagcggatgcacatttacctctcctcacctggcccagagagtggccagcacagtgtatcagaattgcgagcacgccgacaattatactgcctactgcctgggcattagccacatggagcccagctttggcctgatcctgcatgatggcggcacaacactgaaattcgtggatacccccgagagcctgtctggcctgtacgtgttcgtggtgtactttaatggccacgtggaggccgtggcctacacagtggttagcacagtggatcacttcgtgaacgccatcgaagagagaggctttccacctacagccggacagcctcctgctaccacaaaacccaaggagatcacccctgtgaatcctggaaccagcccactgctgagatatgctgcttggacaggcggcctggctgctgtggtgctgctgtgtctggtgatctttctgatctgtaccgctaagaggatgagggtgaaggccgccagagtggataaaagcccatacaaccagagcatgtactacgccggcctgcctgtggatgattttgaggatgctgaagccgccgatgccgaagaggagtttggcaatgccattggcggaagccacggcggcagcagctacaccgtgtacatcgacaagacaaggtatccctacgatgtgcctgattatgccggaagctctggcgtgtctggatggaggctgttcaagaagatcagc

SEQ ID NO: 18 - RNA, 1752 nt, synthetic construct
  source 1..1752: mol_type = other RNA
atgggcaccgtgaataagccagtggtgggcgtgctgatgggctttggcattatcaccggaacactgaggatcaccaacccagtgagggcctctgtgctgagatacgacgacttccacatcgacgaggacaagctggacaccaacagcgtgtacgagccatactaccacagcgatcatgccgagagctcttgggtgaacaggggagagagcagcaggaaggcctacgaccacaattctccctatatctggcccaggaacgactacgatggcttcctggagaatgcccatgaacaccacggagtgtacaaccagggcagaggcattgactctggagagaggctgatgcagccaacccagatgtctgcccaggaggatctgggagacgataccggcatccatgtgattcccacactgaacggagacgacaggcacaagatcgtgaatgtggaccagagacagtacggcgatgtgttcaagggcgacctgaatcctaagcctcagggccagcgactgattgaggtgtctgtggaggagaaccatcctttcacactgcgggctcctatccagcggatctacggcgtgagatacaccgaaacctggagctttctgccaagcctgacctgtacaggcgatgccgctcctgctatccagcacatctgcctgaagcatacaacatgctttcaggacgtggtggtggatgtggattgcgccgagaacaccaaagaggaccagctggccgagattagctacagattccagggcaagaaggaggccgatcagccctggatcgtggtgaatacctctaccctgtttgacgagctggagctggacccccctgagattgagcctggagtgctgaaggtgctgagaacagagaagcagtacctgggcgtgtacatttggaacatgagaggcagcgacggcacctctacctatgccacatttctggtgacctggaagggcgacgagaaaaccagaaatccaacacctgccgtgacaccccagcccaggggagccgagtttcacatgtggaattaccacagccacgtgttcagcgtgggcgacacatttagcctggccatgcacctgcagtacaaaatccacgaggctcctttcgatctgctgctggagtggctgtatgtgcctattgaccctacctgccagcctatgaggctgtacagcacctgtctgtaccacccaaacgcccctcagtgcctgagccatatgaacagcggctgtacattcacctctccacacctggcccagagagtggccagcaccgtgtatcagaattgcgagcatgccgataactacacagcctactgtctgggcattagccacatggagcctagctttggcctgatcctgcacgatggaggcaccaccctgaaattcgtggatacccccgagagcctgagcggcctgtacgtgtttgtggtgtacttcaatggacacgtggaggccgtggcctacacagtggtgagcacagtggatcacttcgtgaacgctattgaggagagaggatttcctccaacagccggccagcctccagccacaaccaaacccaaagaaatcacccccgtgaatcctggaacatctcccctgctgaggtatgctgcttggacaggaggcctggctgccgtggtgctgctgtgcctggtgatctttctgatctgtacctatccatacgatgtgcccgattatgccggatcttctggagtgtctggctggcggctgttcaagaagatcagc

SEQ ID NO: 19 - RNA, 1752 nt, synthetic construct
  source 1..1752: mol_type = other RNA
atgggcaccgtgaacaagcctgtggtgggagtgctgatgggcttcggaatcattacaggcacactgagaatcaccaatcctgtgagagccagcgtgctgcggtacgacgacttccacatcgacgaggacaagctggacaccaacagcgtgtacgagccctactaccacagcgaccacgccgagagcagctgggtgaataggggcgaatctagcagaaaagcctacgaccacaatagcccttacatctggcctaggaacgattacgacggatttctggagaatgctcacgagcaccacggcgtgtacaatcagggcaggggcattgactctggcgagaggctgatgcagcctacccagatgagcgcccaggaagatctgggcgacgacacaggcatccatgtgatccctacactgaatggagacgacagacacaagatcgtgaatgtggatcagagacagtacggcgacgtgtttaaaggcgatctgaaccccaagcctcagggccagcggctgatcgaggtgtctgtggaggagaaccacccttttacactgcgggcccctatccagcggatctacggcgtgagatacacagagacatggagcttcctgccttctctgacctgtacaggagacgctgctcctgccattcagcacatctgcctgaaacacaccacatgctttcaggacgtggtggtggacgtggattgtgccgagaataccaaggaggaccagctggccgagatcagctacaggttccagggaaagaaggaggccgaccagccttggattgtggtgaacacctctaccctgtttgatgagctggagctggaccctccagagattgagcccggcgtgctgaaagtgctgagaaccgagaagcagtatctgggcgtgtatatctggaacatgaggggcagcgatggaaccagcacctacgccaccttcctggtgacatggaagggcgacgagaagacaaggaatcctacaccagccgtgacacctcagccaagaggcgccgagtttcacatgtggaattatcactctcacgtgttcagcgtgggcgacaccttcagcctggccatgcatctgcagtataagatccacgaggccccctttgatctgctgctggagtggctgtatgtgcctatcgacccaacctgccagccaatgaggctgtactctacctgcctgtaccacccaaacgcccctcagtgcctgagccacatgaacagcggctgtacatttacaagcccccatcttgctcagagggtggcctctacagtgtaccagaattgcgagcacgccgataattacacagcctactgcctgggcatcagccacatggagcctagctttggcctgatcctgcacgatggcggcaccaccctgaagtttgtggatacacctgagagcctgagcggcctgtacgtgttcgtggtgtactttaacggacatgtggaggccgtggcctatacagtggtgagcaccgtggaccattttgtgaatgccattgaggagagaggattccctcctacagccggacagcctccagccaccaccaagccaaaggaaatcacacccgtgaatccaggaacctctcctctgctgagatatgctgcctggacaggcggcctggctgctgtggtgctgctgtgtctggttatcttcctgatctgtacatacccttacgatgtgccagattacgccggaagctctggcgtgtctggctggcggctgttcaagaagatcagc

SEQ ID NO: 20 - RNA, 1752 nt, synthetic construct
  source 1..1752: mol_type = other RNA
atgggcaccgtgaataagcccgtggtgggcgtgctgatgggctttggcatcatcacaggaacactgagaatcaccaaccctgtgagagccagcgtgctgagatacgacgactttcacatcgacgaggacaagctggacaccaacagcgtgtacgagccttactaccacagcgaccacgccgagagcagctgggtgaataggggagagagcagcaggaaggcctacgaccacaatagcccatacatctggcccagaaacgattacgatggctttctggaaaacgcccacgagcatcacggagtgtacaatcagggaaggggcattgatagcggcgaaaggctgatgcagcccacccagatgtctgcccaggaggatctgggagatgataccggcattcacgtgatccccaccctgaatggcgacgacaggcacaagatcgtgaacgtggaccagagacagtatggcgacgtgttcaaaggagatctgaaccctaagcctcagggacagaggctgattgaggtgagcgtggaggagaaccacccttttaccctgcgggcccctatccagagaatctacggcgtgagatacaccgaaacatggagcttcctgccttctctgacatgcacaggcgatgccgcccctgccatccagcacatctgcctgaagcacacaacatgctttcaggatgtggtggtggatgtggattgtgccgagaacacaaaggaggaccagctggccgagatctcttacagattccagggcaagaaggaggccgaccagccttggatcgtggtgaatacctctaccctgttcgatgagctggagctggacccaccagagatcgagcctggcgtgctcaaggtgctgagaaccgagaaacagtacctgggcgtgtacatttggaacatgagaggctctgacggcacatctacctacgccacctttctggtgacctggaagggagacgagaagaccagaaacccaacacctgccgtgacaccccagccaagaggcgccgagtttcacatgtggaattatcacagccacgtgttcagcgtgggcgacaccttcagcctggctatgcatctgcagtataagatccacgaagccccattcgacctgctgctggagtggctgtatgtgccaatcgacccaacatgccagcccatgcgcctgtacagcacctgtctgtatcatcctaacgccccacagtgcttaagccacatgaacagcggctgtacattcacatctccacacctcgcccagagggtggccagcaccgtgtaccagaattgtgaacatgccgacaattacaccgcctactgcctgggaatcagccacatggagcctagcttcggcctgatcctgcacgatggaggcacaaccctgaagtttgtggacacacccgagtcactgagcggcctgtacgtgtttgtggtgtacttcaatggacacgtggaggccgtggcctacacagtggtgtctaccgtggatcatttcgtgaacgctatcgaggagagaggatttcctcctacagctggacagcctcccgccaccaccaaacccaaggagattacacctgtgaatccaggcacatctcccctgctgcggtatgctgcttggacaggaggcctggctgctgtggtgctgctgtgtctggtgatcttcctgatctgcacctacccttacgatgtccctgactatgccggctctagcggagtgtctggctggagattgttcaagaagatcagc

SEQ ID NO: 21 - RNA, 1791 nt, synthetic construct
  source 1..1791: mol_type = other RNA
atgggcaccgtgaacaagcctgtggtgggcgtgctgatgggatttggaatcatcaccggcaccctgagaatcaccaaccctgtgagagccagcgtgctgaggtatgacgacttccatatcgacgaggacaagctggacaccaatagcgtgtacgagccctactaccacagcgaccacgccgagagctcttgggtgaatagaggagagagcagcaggaaggcctacgatcacaacagcccttacatctggcccagaaacgactatgacggcttcctggaaaacgcccacgagcaccatggcgtgtataatcagggcagaggaatcgatagcggagagaggctgatgcaacctacccagatgtctgcccaggaggatctgggcgatgataccggaatccacgtgatccctaccctgaacggcgacgacagacacaagatcgtgaatgtggaccagagacagtacggcgatgtgttcaagggcgatctgaaccccaaacctcagggacagaggctcatcgaggtgagcgtggaggagaaccatccttttaccctgagggcccctatccagagaatctacggcgtgaggtataccgagacatggtccttcctgcccagcctgacctgtacaggcgatgccgctcctgccatccagcatatttgcctgaagcataccacctgttttcaggatgtggtggtggatgtggattgcgccgagaacaccaaggaggaccagctggccgagatctcttatagattccagggcaagaaggaggccgaccagccttggattgtggtgaacacctctaccctgttcgacgagctggagctggacccccctgagattgaaccaggcgttctgaaggtgctgagaaccgagaagcagtacctgggagtgtacatctggaatatgagaggcagcgatggcaccagcacctacgctacctttctggtgacctggaagggagacgagaaaaccaggaatccaacccctgccgtgacaccacagcccagaggcgccgagtttcacatgtggaattaccacagccacgtgttcagcgtgggcgacaccttctctctggccatgcacctgcagtataagattcacgaagctccatttgacctgctgctggagtggctgtacgtgccaattgaccccacatgccagccaatgaggctgtacagcacctgcctgtaccatccaaacgccccccagtgcctgtctcacatgaacagcggctgtacatttacaagccctcacctggcccagcgagtggccagcacagtgtaccagaattgtgagcatgctgacaattacacagcctattgcctgggcatcagccacatggagccatctttcggcctgatcctgcacgatggcggcaccaccctgaaatttgtggatacccctgagagcctgagcggcctgtacgtgtttgtggtgtactttaacggccacgtggaggccgtggcctacaccgtggtgagcacagtggatcattttgtgaatgccatcgaagaaagaggcttccctcctacagccggacagcctcctgccacaacaaagcccaaggagattaccccagtgaatccaggaacctctccactgctgagatacgccgcttggacaggaggcctggctgctgtggtgctgctgtgcctggtgatcttcctgatttgcaccgctaagagaatgagagtgaaagccgccagagtggataagtacccttacgacgtgcccgattatgctggaagctctggagtgtctggctggaggctgttcaagaagatcagc

SEQ ID NO: 22 - RNA, 1791 nt, synthetic construct
  source 1..1791: mol_type = other RNA
atgggcaccgtgaacaagcctgtggtgggcgtgctcatgggctttggcatcatcacaggcaccctgagaatcaccaatcccgtgagagccagcgtgctgcggtacgacgacttccacatcgacgaggacaagctggacaccaatagcgtgtacgagccctactaccacagcgaccacgccgagagcagctgggtgaatagaggagaatctagcaggaaggcctatgaccacaatagcccatacatttggcccaggaatgattacgacggcttcctggagaacgcccacgagcaccacggcgtgtacaaccagggaagaggcattgattctggcgaacggctgatgcagccaacacagatgagcgcccaggaggacctgggagatgataccggaatccacgtgattcctaccctgaacggcgatgatagacacaagatcgtgaacgtggaccagagacagtacggcgacgtgtttaagggcgacctgaaccccaagcctcagggacagaggctgattgaggtgagcgtggaagagaaccaccctttcacactgagagcccccatccagaggatttacggcgtgaggtacacagagacatggagctttctgcctagcctgacatgtacaggcgatgccgcccctgccattcagcacatctgcctgaagcacaccacctgttttcaggatgtggtggtggatgtggattgcgccgagaacaccaaggaggatcagctggccgagatcagctacagattccagggaaagaaggaggccgaccagccttggatcgtggtgaatacaagcaccctgttcgatgagctggagctggaccctcccgagattgaacctggcgtgctgaaggtgctgaggaccgagaagcagtatctgggagtgtacatttggaatatgaggggcagcgacggcacatctacctacgccaccttcctggtgacatggaagggcgacgaaaaaacccggaatcctacccctgccgtgaccccacagcctagaggagccgagtttcacatgtggaattaccacagccacgtgttcagcgtgggagacacattctctctggccatgcacctgcagtacaagattcacgaagccccattcgacctgctgctggagtggctgtatgtgcccattgatcccacctgtcagcccatgcgactgtacagcacctgtctgtatcacccaaacgccccccagtgtctgtctcacatgaatagcggatgcacctttacaagcccacatctggcccagagggtggctagcacagtgtaccagaattgcgagcacgccgacaactacacagcttactgcctgggcatcagccacatggagccttctttcggcctgatcctgcacgacggcggcacaacactgaaatttgtggataccccagagagcctgtctggcctgtacgtgtttgtggtgtattttaacggccacgtggaggccgtggcctacacagtggtgtctaccgtggaccactttgtgaacgctatcgaggagagaggctttcctccaacagctggacagcctccagctaccacaaagcctaaggagatcacccctgtgaaccccggaacatctccactgctgagatacgccgcttggaccggcggattggctgccgttgtgctgctgtgcctggtgatctttctgatttgtacagccaagagaatgagagtgaaggctgctcgggtggacaagtatccatacgatgtgcccgattatgccggatcttctggcgtgagcggctggagattgttcaagaagatctcc

SEQ ID NO: 23 - RNA, 1791 nt, synthetic construct
  source 1..1791: mol_type = other RNA
atgggcaccgtgaacaagcctgtggtgggagtgctcatgggatttggaatcattacaggcacactgaggatcaccaaccccgtgagagccagcgtgctgaggtacgatgacttccacatcgacgaggacaagctggacaccaacagcgtgtacgagccctactaccacagcgaccacgccgagagctcttgggtgaataggggcgaatctagcagaaaggcctacgaccacaatagcccctatatttggcctagaaacgactacgatggcttcctggagaacgcccacgagcaccacggagtgtacaatcagggcagaggcatcgatagcggcgaaaggctgatgcagcctacccagatgagcgcccaggaagatctgggcgatgacacaggcatccatgtgattcctacactgaacggcgacgacaggcacaaaatcgtgaatgtggatcagaggcagtacggcgacgtgtttaagggcgatctgaatcccaagccacagggccagaggctgatcgaagtgagcgtggaggagaatcacccttttaccctgcgggccccaatccagcggatctacggagtgaggtataccgaaacatggagctttctgccaagcctgacctgtaccggagacgctgcccctgctatccagcacatttgtctgaagcacaccacctgttttcaggacgtggtggtggatgtggattgtgccgagaacaccaaggaggaccagctggccgagatcagctacagattccagggcaagaaggaggccgatcagccatggattgttgtgaataccagcaccctgttcgacgagctggagctggaccctccagaaattgagcctggcgtgctgaaggtgctgagaaccgagaaacagtacctgggagtttacatctggaacatgaggggctccgacggcacaagcacctacgctaccttcctggtgacatggaagggcgacgagaagacaagaaatcctaccccagccgtgacaccacagcccaggggcgccgagtttcatatgtggaattaccacagccacgtgttcagcgtgggcgatacatttagcctggccatgcatctgcagtacaagatccacgaggctcctttcgacctgctgctggaatggctgtacgtgccaatcgaccccacatgccagcctatgaggctgtatagcacatgcctgtatcaccctaacgccccccagtgcctgagccacatgaacagcggatgcacatttacctctcctcacctggcccagagagtggccagcacagtgtatcagaattgcgagcacgccgacaattatactgcctactgcctgggcattagccacatggagcccagctttggcctgatcctgcatgatggcggcacaacactgaaattcgtggatacccccgagagcctgtctggcctgtacgtgttcgtggtgtactttaatggccacgtggaggccgtggcctacacagtggttagcacagtggatcacttcgtgaacgccatcgaagagagaggctttccacctacagccggacagcctcctgctaccacaaaacccaaggagatcacccctgtgaatcctggaaccagcccactgctgagatatgctgcttggacaggcggcctggctgctgtggtgctgctgtgtctggtgatctttctgatctgtaccgctaagaggatgagggtgaaggccgccagagtggataaatatccctacgatgtgcctgattatgccggaagctctggcgtgtctggatggaggctgttcaagaagatcagc

SEQ ID NO: 24 - RNA, 1941 nt, synthetic construct
  source 1..1941: mol_type = other RNA
atgggcaccgtgaacaagcctgtggtgggcgtgctgatgggatttggaatcatcaccggcaccctgagaatcaccaaccctgtgagagccagcgtgctgaggtatgacgacttccatatcgacgaggacaagctggacaccaatagcgtgtacgagccctactaccacagcgaccacgccgagagctcttgggtgaatagaggagagagcagcaggaaggcctacgatcacaacagcccttacatctggcccagaaacgactatgacggcttcctggaaaacgcccacgagcaccatggcgtgtataatcagggcagaggaatcgatagcggagagaggctgatgcaacctacccagatgtctgcccaggaggatctgggcgatgataccggaatccacgtgatccctaccctgaacggcgacgacagacacaagatcgtgaatgtggaccagagacagtacggcgatgtgttcaagggcgatctgaaccccaaacctcagggacagaggctcatcgaggtgagcgtggaggagaaccatccttttaccctgagggcccctatccagagaatctacggcgtgaggtataccgagacatggtccttcctgcccagcctgacctgtacaggcgatgccgctcctgccatccagcatatttgcctgaagcataccacctgttttcaggatgtggtggtggatgtggattgcgccgagaacaccaaggaggaccagctggccgagatctcttatagattccagggcaagaaggaggccgaccagccttggattgtggtgaacacctctaccctgttcgacgagctggagctggacccccctgagattgaaccaggcgttctgaaggtgctgagaaccgagaagcagtacctgggagtgtacatctggaatatgagaggcagcgatggcaccagcacctacgctacctttctggtgacctggaagggagacgagaaaaccaggaatccaacccctgccgtgacaccacagcccagaggcgccgagtttcacatgtggaattaccacagccacgtgttcagcgtgggcgacaccttctctctggccatgcacctgcagtataagattcacgaagctccatttgacctgctgctggagtggctgtacgtgccaattgaccccacatgccagccaatgaggctgtacagcacctgcctgtaccatccaaacgccccccagtgcctgtctcacatgaacagcggctgtacatttacaagccctcacctggcccagcgagtggccagcacagtgtaccagaattgtgagcatgctgacaattacacagcctattgcctgggcatcagccacatggagccatctttcggcctgatcctgcacgatggcggcaccaccctgaaatttgtggatacccctgagagcctgagcggcctgtacgtgtttgtggtgtactttaacggccacgtggaggccgtggcctacaccgtggtgagcacagtggatcattttgtgaatgccatcgaagaaagaggcttccctcctacagccggacagcctcctgccacaacaaagcccaaggagattaccccagtgaatccaggaacctctccactgctgagatacgccgcttggacaggaggcctggctgctgtggtgctgctgtgcctggtgatcttcctgatttgcaccgctaagagaatgagagtgaaagccgccagagtggataagagcccctacaaccagagcatgtacggcgccggcctgcctgtggatgatttcgaagatgccgaagctgccgatgctgaggaggagtttggcaatgccattggcggcagccacggcggcagcagctataccgtgtacatcgacaagacaaggtacccttacgacgtgcccgattatgctggaagctctggagtgtctggctggaggctgttcaagaagatcagc

SEQ ID NO: 25 - RNA, 1941 nt, synthetic construct
  source 1..1941: mol_type = other RNA
atgggcaccgtgaacaagcctgtggtgggcgtgctcatgggctttggcatcatcacaggcaccctgagaatcaccaatcccgtgagagccagcgtgctgcggtacgacgacttccacatcgacgaggacaagctggacaccaatagcgtgtacgagccctactaccacagcgaccacgccgagagcagctgggtgaatagaggagaatctagcaggaaggcctatgaccacaatagcccatacatttggcccaggaatgattacgacggcttcctggagaacgcccacgagcaccacggcgtgtacaaccagggaagaggcattgattctggcgaacggctgatgcagccaacacagatgagcgcccaggaggacctgggagatgataccggaatccacgtgattcctaccctgaacggcgatgatagacacaagatcgtgaacgtggaccagagacagtacggcgacgtgtttaagggcgacctgaaccccaagcctcagggacagaggctgattgaggtgagcgtggaagagaaccaccctttcacactgagagcccccatccagaggatttacggcgtgaggtacacagagacatggagctttctgcctagcctgacatgtacaggcgatgccgcccctgccattcagcacatctgcctgaagcacaccacctgttttcaggatgtggtggtggatgtggattgcgccgagaacaccaaggaggatcagctggccgagatcagctacagattccagggaaagaaggaggccgaccagccttggatcgtggtgaatacaagcaccctgttcgatgagctggagctggaccctcccgagattgaacctggcgtgctgaaggtgctgaggaccgagaagcagtatctgggagtgtacatttggaatatgaggggcagcgacggcacatctacctacgccaccttcctggtgacatggaagggcgacgaaaaaacccggaatcctacccctgccgtgaccccacagcctagaggagccgagtttcacatgtggaattaccacagccacgtgttcagcgtgggagacacattctctctggccatgcacctgcagtacaagattcacgaagccccattcgacctgctgctggagtggctgtatgtgcccattgatcccacctgtcagcccatgcgactgtacagcacctgtctgtatcacccaaacgccccccagtgtctgtctcacatgaatagcggatgcacctttacaagcccacatctggcccagagggtggctagcacagtgtaccagaattgcgagcacgccgacaactacacagcttactgcctgggcatcagccacatggagccttctttcggcctgatcctgcacgacggcggcacaacactgaaatttgtggataccccagagagcctgtctggcctgtacgtgtttgtggtgtattttaacggccacgtggaggccgtggcctacacagtggtgtctaccgtggaccactttgtgaacgctatcgaggagagaggctttcctccaacagctggacagcctccagctaccacaaagcctaaggagatcacccctgtgaaccccggaacatctccactgctgagatacgccgcttggaccggcggattggctgccgttgtgctgctgtgcctggtgatctttctgatttgtacagccaagagaatgagagtgaaggctgctcgggtggacaagagcccttacaatcagagcatgtacggcgccggcctgcctgtggatgacttcgaagatgccgaagctgccgatgccgaggaggaatttggcaatgctatcggcggcagccatggcggcagcagctacaccgtgtacatcgacaaaaccaggtatccatacgatgtgcccgattatgccggatcttctggcgtgagcggctggagattgttcaagaagatctcc

SEQ ID NO: 26 - RNA, 1941 nt, synthetic construct
  source 1..1941: mol_type = other RNA
atgggcaccgtgaacaagcctgtggtgggagtgctcatgggatttggaatcattacaggcacactgaggatcaccaaccccgtgagagccagcgtgctgaggtacgatgacttccacatcgacgaggacaagctggacaccaacagcgtgtacgagccctactaccacagcgaccacgccgagagctcttgggtgaataggggcgaatctagcagaaaggcctacgaccacaatagcccctatatttggcctagaaacgactacgatggcttcctggagaacgcccacgagcaccacggagtgtacaatcagggcagaggcatcgatagcggcgaaaggctgatgcagcctacccagatgagcgcccaggaagatctgggcgatgacacaggcatccatgtgattcctacactgaacggcgacgacaggcacaaaatcgtgaatgtggatcagaggcagtacggcgacgtgtttaagggcgatctgaatcccaagccacagggccagaggctgatcgaagtgagcgtggaggagaatcacccttttaccctgcgggccccaatccagcggatctacggagtgaggtataccgaaacatggagctttctgccaagcctgacctgtaccggagacgctgcccctgctatccagcacatttgtctgaagcacaccacctgttttcaggacgtggtggtggatgtggattgtgccgagaacaccaaggaggaccagctggccgagatcagctacagattccagggcaagaaggaggccgatcagccatggattgttgtgaataccagcaccctgttcgacgagctggagctggaccctccagaaattgagcctggcgtgctgaaggtgctgagaaccgagaaacagtacctgggagtttacatctggaacatgaggggctccgacggcacaagcacctacgctaccttcctggtgacatggaagggcgacgagaagacaagaaatcctaccccagccgtgacaccacagcccaggggcgccgagtttcatatgtggaattaccacagccacgtgttcagcgtgggcgatacatttagcctggccatgcatctgcagtacaagatccacgaggctcctttcgacctgctgctggaatggctgtacgtgccaatcgaccccacatgccagcctatgaggctgtatagcacatgcctgtatcaccctaacgccccccagtgcctgagccacatgaacagcggatgcacatttacctctcctcacctggcccagagagtggccagcacagtgtatcagaattgcgagcacgccgacaattatactgcctactgcctgggcattagccacatggagcccagctttggcctgatcctgcatgatggcggcacaacactgaaattcgtggatacccccgagagcctgtctggcctgtacgtgttcgtggtgtactttaatggccacgtggaggccgtggcctacacagtggttagcacagtggatcacttcgtgaacgccatcgaagagagaggctttccacctacagccggacagcctcctgctaccacaaaacccaaggagatcacccctgtgaatcctggaaccagcccactgctgagatatgctgcttggacaggcggcctggctgctgtggtgctgctgtgtctggtgatctttctgatctgtaccgctaagaggatgagggtgaaggccgccagagtggataaaagcccatacaaccagagcatgggctacgccggcctgcctgtggatgattttgaggatgctgaagccgccgatgccgaagaggagtttggcaatgccattggcggaagccacggcggcagcagctacaccgtgtacatcgacaagacaaggtatccctacgatgtgcctgattatgccggaagctctggcgtgtctggatggaggctgttcaagaagatcagc

SEQ ID NO: 27 - RNA, 1869 nt, synthetic construct
  source 1..1869: mol_type = other RNA
atgggcaccgtgaacaagcctgtggtgggcgtgctgatgggatttggaatcatcaccggcaccctgagaatcaccaaccctgtgagagccagcgtgctgaggtatgacgacttccatatcgacgaggacaagctggacaccaatagcgtgtacgagccctactaccacagcgaccacgccgagagctcttgggtgaatagaggagagagcagcaggaaggcctacgatcacaacagcccttacatctggcccagaaacgactatgacggcttcctggaaaacgcccacgagcaccatggcgtgtataatcagggcagaggaatcgatagcggagagaggctgatgcaacctacccagatgtctgcccaggaggatctgggcgatgataccggaatccacgtgatccctaccctgaacggcgacgacagacacaagatcgtgaatgtggaccagagacagtacggcgatgtgttcaagggcgatctgaaccccaaacctcagggacagaggctcatcgaggtgagcgtggaggagaaccatccttttaccctgagggcccctatccagagaatctacggcgtgaggtataccgagacatggtccttcctgcccagcctgacctgtacaggcgatgccgctcctgccatccagcatatttgcctgaagcataccacctgttttcaggatgtggtggtggatgtggattgcgccgagaacaccaaggaggaccagctggccgagatctcttatagattccagggcaagaaggaggccgaccagccttggattgtggtgaacacctctaccctgttcgacgagctggagctggacccccctgagattgaaccaggcgttctgaaggtgctgagaaccgagaagcagtacctgggagtgtacatctggaatatgagaggcagcgatggcaccagcacctacgctacctttctggtgacctggaagggagacgagaaaaccaggaatccaacccctgccgtgacaccacagcccagaggcgccgagtttcacatgtggaattaccacagccacgtgttcagcgtgggcgacaccttctctctggccatgcacctgcagtataagattcacgaagctccatttgacctgctgctggagtggctgtacgtgccaattgaccccacatgccagccaatgaggctgtacagcacctgcctgtaccatccaaacgccccccagtgcctgtctcacatgaacagcggctgtacatttacaagccctcacctggcccagcgagtggccagcacagtgtaccagaattgtgagcatgctgacaattacacagcctattgcctgggcatcagccacatggagccatctttcggcctgatcctgcacgatggcggcaccaccctgaaatttgtggatacccctgagagcctgagcggcctgtacgtgtttgtggtgtactttaacggccacgtggaggccgtggcctacaccgtggtgagcacagtggatcattttgtgaatgccatcgaagaaagaggcttccctcctacagccggacagcctcctgccacaacaaagcccaaggagattaccccagtgaatccaggaacctctccactgctgagatacgccgcttggacaggaggcctggctgctgtggtgctgctgtgcctggtgatcttcctgatttgcaccgctaagagaatgagagtgaaagccgccagagtggataagagcccctacaaccagagcatgtacggcgccggcctgcctgtggatgatttcgaagatgccgaagctgccgatgctgaggaggagtttggcaatgccattggcggcagccacggcggcagcagctataccgtgtacatcgacaagacaagg

SEQ ID NO: 28 - RNA, 1776 nt, synthetic construct
  source 1..1776: mol_type = other RNA
atgggcaccgtgaataagccagtggtgggcgtgctgatgggctttggcattatcaccggaacactgaggatcaccaacccagtgagggcctctgtgctgagatacgacgacttccacatcgacgaggacaagctggacaccaacagcgtgtacgagccatactaccacagcgatcatgccgagagctcttgggtgaacaggggagagagcagcaggaaggcctacgaccacaattctccctatatctggcccaggaacgactacgatggcttcctggagaatgcccatgaacaccacggagtgtacaaccagggcagaggcattgactctggagagaggctgatgcagccaacccagatgtctgcccaggaggatctgggagacgataccggcatccatgtgattcccacactgaacggagacgacaggcacaagatcgtgaatgtggaccagagacagtacggcgatgtgttcaagggcgacctgaatcctaagcctcagggccagcgactgattgaggtgtctgtggaggagaaccatcctttcacactgcgggctcctatccagcggatctacggcgtgagatacaccgaaacctggagctttctgccaagcctgacctgtacaggcgatgccgctcctgctatccagcacatctgcctgaagcatacaacatgctttcaggacgtggtggtggatgtggattgcgccgagaacaccaaagaggaccagctggccgagattagctacagattccagggcaagaaggaggccgatcagccctggatcgtggtgaatacctctaccctgtttgacgagctggagctggacccccctgagattgagcctggagtgctgaaggtgctgagaacagagaagcagtacctgggcgtgtacatttggaacatgagaggcagcgacggcacctctacctatgccacatttctggtgacctggaagggcgacgagaaaaccagaaatccaacacctgccgtgacaccccagcccaggggagccgagtttcacatgtggaattaccacagccacgtgttcagcgtgggcgacacatttagcctggccatgcacctgcagtacaaaatccacgaggctcctttcgatctgctgctggagtggctgtatgtgcctattgaccctacctgccagcctatgaggctgtacagcacctgtctgtaccacccaaacgcccctcagtgcctgagccatatgaacagcggctgtacattcacctctccacacctggcccagagagtggccagcaccgtgtatcagaattgcgagcatgccgataactacacagcctactgtctgggcattagccacatggagcctagctttggcctgatcctgcacgatggaggcaccaccctgaaattcgtggatacccccgagagcctgagcggcctgtacgtgtttgtggtgtacttcaatggacacgtggaggccgtggcctacacagtggtgagcacagtggatcacttcgtgaacgctattgaggagagaggatttcctccaacagccggccagcctccagccacaaccaaacccaaagaaatcacccccgtgaatcctggaacatctcccctgctgaggtatgctgcttggacaggaggcctggctgccgtggtgctgctgtgcctggtgatctttctgatctgtaccgctaagagaatgagggtgaaggcctatccatacgatgtgcccgattatgccggatcttctggagtgtctggctggcggctgttcaagaagatcagc

SEQ ID NO: 29 - RNA, 1776 nt, synthetic construct
  source 1..1776: mol_type = other RNA
atgggcaccgtgaacaagcctgtggtgggagtgctgatgggcttcggaatcattacaggcacactgagaatcaccaatcctgtgagagccagcgtgctgcggtacgacgacttccacatcgacgaggacaagctggacaccaacagcgtgtacgagccctactaccacagcgaccacgccgagagcagctgggtgaataggggcgaatctagcagaaaagcctacgaccacaatagcccttacatctggcctaggaacgattacgacggatttctggagaatgctcacgagcaccacggcgtgtacaatcagggcaggggcattgactctggcgagaggctgatgcagcctacccagatgagcgcccaggaagatctgggcgacgacacaggcatccatgtgatccctacactgaatggagacgacagacacaagatcgtgaatgtggatcagagacagtacggcgacgtgtttaaaggcgatctgaaccccaagcctcagggccagcggctgatcgaggtgtctgtggaggagaaccacccttttacactgcgggcccctatccagcggatctacggcgtgagatacacagagacatggagcttcctgccttctctgacctgtacaggagacgctgctcctgccattcagcacatctgcctgaaacacaccacatgctttcaggacgtggtggtggacgtggattgtgccgagaataccaaggaggaccagctggccgagatcagctacaggttccagggaaagaaggaggccgaccagccttggattgtggtgaacacctctaccctgtttgatgagctggagctggaccctccagagattgagcccggcgtgctgaaagtgctgagaaccgagaagcagtatctgggcgtgtatatctggaacatgaggggcagcgatggaaccagcacctacgccaccttcctggtgacatggaagggcgacgagaagacaaggaatcctacaccagccgtgacacctcagccaagaggcgccgagtttcacatgtggaattatcactctcacgtgttcagcgtgggcgacaccttcagcctggccatgcatctgcagtataagatccacgaggccccctttgatctgctgctggagtggctgtatgtgcctatcgacccaacctgccagccaatgaggctgtactctacctgcctgtaccacccaaacgcccctcagtgcctgagccacatgaacagcggctgtacatttacaagcccccatcttgctcagagggtggcctctacagtgtaccagaattgcgagcacgccgataattacacagcctactgcctgggcatcagccacatggagcctagctttggcctgatcctgcacgatggcggcaccaccctgaagtttgtggatacacctgagagcctgagcggcctgtacgtgttcgtggtgtactttaacggacatgtggaggccgtggcctatacagtggtgagcaccgtggaccattttgtgaatgccattgaggagagaggattccctcctacagccggacagcctccagccaccaccaagccaaaggaaatcacacccgtgaatccaggaacctctcctctgctgagatatgctgcctggacaggcggcctggctgctgtggtgctgctgtgtctggttatcttcctgatctgtacagctaagaggatgcgggtgaaggcctacccttacgatgtgccagattacgccggaagctctggcgtgtctggctggcggctgttcaagaagatcagc

SEQ ID NO: 30 - RNA, 1776 nt, synthetic construct
  source 1..1776: mol_type = other RNA
atgggcaccgtgaataagcccgtggtgggcgtgctgatgggctttggcatcatcacaggaacactgagaatcaccaaccctgtgagagccagcgtgctgagatacgacgactttcacatcgacgaggacaagctggacaccaacagcgtgtacgagccttactaccacagcgaccacgccgagagcagctgggtgaataggggagagagcagcaggaaggcctacgaccacaatagcccatacatctggcccagaaacgattacgatggctttctggaaaacgcccacgagcatcacggagtgtacaatcagggaaggggcattgatagcggcgaaaggctgatgcagcccacccagatgtctgcccaggaggatctgggagatgataccggcattcacgtgatccccaccctgaatggcgacgacaggcacaagatcgtgaacgtggaccagagacagtatggcgacgtgttcaaaggagatctgaaccctaagcctcagggacagaggctgattgaggtgagcgtggaggagaaccacccttttaccctgcgggcccctatccagagaatctacggcgtgagatacaccgaaacatggagcttcctgccttctctgacatgcacaggcgatgccgcccctgccatccagcacatctgcctgaagcacacaacatgctttcaggatgtggtggtggatgtggattgtgccgagaacacaaaggaggaccagctggccgagatctcttacagattccagggcaagaaggaggccgaccagccttggatcgtggtgaatacctctaccctgttcgatgagctggagctggacccaccagagatcgagcctggcgtgctcaaggtgctgagaaccgagaaacagtacctgggcgtgtacatttggaacatgagaggctctgacggcacatctacctacgccacctttctggtgacctggaagggagacgagaagaccagaaacccaacacctgccgtgacaccccagccaagaggcgccgagtttcacatgtggaattatcacagccacgtgttcagcgtgggcgacaccttcagcctggctatgcatctgcagtataagatccacgaagccccattcgacctgctgctggagtggctgtatgtgccaatcgacccaacatgccagcccatgcgcctgtacagcacctgtctgtatcatcctaacgccccacagtgcttaagccacatgaacagcggctgtacattcacatctccacacctcgcccagagggtggccagcaccgtgtaccagaattgtgaacatgccgacaattacaccgcctactgcctgggaatcagccacatggagcctagcttcggcctgatcctgcacgatggaggcacaaccctgaagtttgtggacacacccgagtcactgagcggcctgtacgtgtttgtggtgtacttcaatggacacgtggaggccgtggcctacacagtggtgtctaccgtggatcatttcgtgaacgctatcgaggagagaggatttcctcctacagctggacagcctcccgccaccaccaaacccaaggagattacacctgtgaatccaggcacatctcccctgctgcggtatgctgcttggacaggaggcctggctgctgtggtgctgctgtgtctggtgatcttcctgatctgcaccgctaaaagaatgagggtgaaagcctacccttacgatgtccctgactatgccggctctagcggagtgtctggctggagattgttcaagaagatcagc

SEQ ID NO: 31 - RNA, 1725 nt, synthetic construct
  source 1..1725: mol_type = other RNA
atgggcaccgtgaacaagcctgtggtgggcgtgctgatgggctttggcatcatcacaggcacactgaggatcaccaatcccgtgagagcctctgtgctgagatacgacgacttccacatcgacgaggacaagctggacaccaactctgtgtacgagccctactaccacagcgatcacgccgaaagcagctgggtgaatagaggcgagagcagcagaaaggcctacgatcacaacagcccctacatctggcctaggaacgactacgacggatttctggagaacgcccacgagcatcacggagtgtacaatcagggcagaggcattgatagcggcgagaggctgatgcagcctacacagatgtctgctcaggaggatctgggagacgataccggcattcacgtgatccctaccctgaacggcgacgacagacacaagatcgtgaacgtggaccagagacagtacggcgacgtgtttaagggcgatctgaatcctaaacctcagggccagcggctgatcgaagtgagcgtggaggagaatcaccctttcaccctgagagcccccatccagagaatctacggcgtgagatacaccgaaacctggagctttctgcccagcctgacatgtaccggagatgccgctcctgccatccagcacatctgtctgaagcacacaacctgctttcaggacgtggtggtggatgtggattgtgccgagaataccaaggaggaccagctggccgagatcagctacagattccagggcaagaaagaggccgatcagccttggatcgtggtgaataccagcaccctgttcgatgagctggagctggaccctcctgagatcgaaccaggagtgctgaaggtgctgaggaccgagaaacagtacctgggcgtgtacatctggaacatgagaggctctgatggcacctctacctacgccacattcctggtgacctggaagggcgatgagaagacaaggaacccaacacctgccgtgacaccacagccaaggggcgccgagtttcacatgtggaattaccactctcacgtgttcagcgtgggcgacacattcagcctggccatgcacctgcagtataagattcacgaggctcctttcgatctgctgctggagtggctgtacgtgcctatcgatcctacctgccagccaatgaggctgtacagcacctgcctgtaccacccaaatgctccccagtgcctgagccacatgaatagcggctgtacattcacaagcccacacctggcccagagagtggcctctaccgtgtaccagaattgtgagcatgccgacaattacacagcctactgtctgggcatcagccacatggagccatccttcggcctgatcctgcatgacggcggcacaacactgaagtttgtggacacccctgaaagcctgagcggcctgtatgtgttcgtggtgtacttcaatggccacgtggaggccgtggcctataccgtggtgtctaccgtggatcactttgtgaacgccattgaggaaagaggatttcctcctacagccggacagcctcctgccaccaccaagcctaaggagatcaccccagtgaatccaggaaccagccctctgctgagacagatcctggccatttacagcacagtggcttctagcctggtgctggtggtgagcctgggcgccatctctttttggatgtgcagcaatggcagcctgcagtgcagaatctgcatc

SEQ ID NO: 32 - RNA, 1725 nt, synthetic construct
  source 1..1725: mol_type = other RNA
atgggcaccgtgaacaagcctgtggtgggcgtgctgatgggctttggcatcatcacaggcacactgaggatcaccaatcccgtgagagccagcgtgctgaggtacgacgacttccacatcgacgaggacaagctggacacaaactctgtgtacgagccctactaccacagcgatcacgccgaaagcagctgggtgaatagaggcgagagcagcagaaaggcctacgatcacaacagcccctacatctggcctaggaatgactacgacggattcctggagaacgcccacgagcatcacggagtgtacaatcagggcagaggcattgatagcggcgagaggctgatgcagcctacacagatgtctgctcaggaggatctgggagacgataccggcattcacgtgatccctaccctgaacggcgacgacagacacaagatcgtgaacgtggaccagagacagtacggcgacgtgtttaagggcgatctgaatcctaaacctcagggccagcggctgatcgaagtgagcgtggaggagaatcaccctttcaccctgagagcccccatccagagaatctacggcgtgagatacaccgaaacctggagctttctgcccagcctgacatgtaccggagatgccgctcctgccatccagcacatctgtctgaagcacacaacctgctttcaggacgtggtggtggatgtggattgtgccgagaataccaaggaggaccagctggccgagatcagctacagattccagggcaagaaggaggccgatcagccatggattgtggtgaataccagcaccctgttcgatgagctggagctggaccctcctgagatcgagccaggagtgctgaaggtgctgaggaccgaaaaacagtacctgggcgtgtacatctggaatatgaggggctctgatggcacctctacctacgccacattcctggtgacctggaagggcgatgagaagacaaggaacccaacacctgccgtgacaccacagccaaggggcgccgagtttcacatgtggaattaccactctcacgtgttcagcgtgggcgacacattcagcctggccatgcacctgcagtataagattcacgaggctcctttcgatctgctgctggagtggctgtacgtgcccatcgatcctacctgtcagccaatgaggctgtacagcacctgcctgtaccacccaaatgccccccagtgcctgagccatatgaacagcggctgtacatttacaagcccacacctggcccagagagtggcctctaccgtgtaccagaattgtgagcatgccgacaattacacagcctactgtctgggcatcagccacatggagccatccttcggcctgatcctgcatgacggcggcacaacactgaagtttgtggacacccctgaaagcctgagcggcctgtatgtgttcgtggtgtacttcaatggccacgtggaggccgtggcctataccgtggtgtctaccgtggatcactttgtgaacgccattgaggaaagaggatttcctcctacagccggacagcctcctgccaccaccaagcctaaggagatcacacccgtgaatccaggaaccagccctctgctgaggcagattctggccatttacagcacagtggcttctagcctggtgctggtggtgagcctgggcgccatctctttttggatgtgcagcaacggcagcctgcagtgtagaatctgcatc

SEQ ID NO: 33 - RNA, 1725 nt, synthetic construct
  source 1..1725: mol_type = other RNA
atgggcaccgtgaacaagcctgtggtgggcgtgctgatgggctttggaatcatcacaggcacactgaggatcaccaatcccgtgagagccagcgtgctgaggtacgacgacttccacatcgacgaggacaagctggacacaaactctgtgtacgagccctactaccacagcgatcacgccgaaagcagctgggtgaatagaggcgagagcagcagaaaggcctacgatcacaacagcccctacatctggcctaggaatgactacgacggattcctggaaaacgcccacgagcaccacggagtgtacaatcagggcagaggcattgatagcggcgagaggctgatgcagcctacacagatgtctgctcaggaagatctgggagacgacaccggcattcacgtgatccctaccctgaacggcgacgatagacacaagatcgtgaacgtggaccagaggcagtatggcgacgtgtttaagggcgacctgaatcctaagcctcagggacagcggctgattgaagtgagcgtggaggagaaccacccattcaccctgagagccccaatccagagaatctacggcgtgagatacaccgaaacctggagcttcctgcccagcctgacatgcaccggagatgcagctcctgctatccagcacatctgcctgaagcacacaacctgtttccaggatgttgtggttgatgtggattgcgccgagaacaccaaggaggaccagctggccgagatcagctacagattccagggcaagaaggaggccgatcagccatggattgtggtgaataccagcaccctgttcgatgagctggagctggaccctcctgagatcgagccaggagtgctgaaggtgctgaggaccgaaaagcagtacctgggcgtgtatatctggaatatgaggggctctgatggcacctctacctacgccacattcctggtgacctggaagggcgatgagaaaacaaggaaccctacacctgccgtgacaccacagcccaggggcgccgagtttcacatgtggaattaccactctcacgtgttcagcgtgggcgacacatttagcctggccatgcacctgcagtacaaaattcacgaggctcccttcgatctgctgctggagtggctgtatgtgcccatcgatcccacctgtcagccaatgaggctgtatagcacatgcctgtaccacccaaacgccccccagtgcctgagccatatgaatagcggctgcacatttacaagcccacacctggcccagagagtggccagtaccgtgtaccagaattgtgagcatgccgataactacacagcctactgtctgggcatcagccacatggagccatccttcggcctgatcctgcacgacggcggcacaacactgaagtttgtggacacacccgagagcctgagcggcctgtatgtgtttgtggtgtactttaatggccacgtggaggctgtggcctacaccgtggtgtctacagtggatcactttgtgaatgccatcgaggaaagaggattccctcctacagccggacagcctcctgccaccaccaaacccaaggagatcacacccgtgaatccaggcaccagccctctgctgaggcagattctggccatttatagtacagtggcttctagcctggtgctggtggtgagcctgggcgccatctctttttggatgtgtagcaacggcagcctgcagtgtagaatctgcatc

SEQ ID NO: 34 - RNA, 1743 nt, synthetic construct
  source 1..1743: mol_type = other RNA
atgggcaccgtgaataagcccgtggtgggcgtgctgatgggctttggcatcatcacaggcaccctgaggatcaccaatccagtgagagcctctgtgctgaggtacgacgacttccacatcgatgaggacaagctggacaccaatagcgtgtacgagccctactaccacagcgatcatgccgagagcagctgggtgaatagaggagagagcagcagaaaggcctacgaccacaacagcccctacatctggcccaggaacgactacgatggcttcctggagaatgcccacgaacatcacggcgtgtacaaccagggaagaggcatcgattctggagaaaggctgatgcagcctacccagatgtctgcccaggaggatctgggcgatgatacaggaatccatgtgatccctaccctgaacggcgacgacaggcacaagatcgtgaacgtggaccagaggcagtatggcgacgtgttcaagggcgacctgaatcctaagcctcagggacagaggctgattgaggtgagcgtggaagagaatcaccctttcaccctgagagcccctatccagaggatctacggcgtgaggtatacagagacatggagcttcctgccttctctgacctgtaccggagatgccgcccctgccattcagcacatctgcctgaaacacaccacctgctttcaggacgtggtggtggatgttgactgtgccgagaacaccaaggaggatcagctggccgaaatcagctacaggttccagggcaagaaagaggccgatcagccttggattgtggtgaacaccagcaccctgtttgatgagctggagctggaccctcctgagatcgagcctggagtgctgaaggtgctgaggaccgagaagcagtacctgggagtgtacatctggaatatgaggggctctgacggcacaagcacatatgccaccttcctggtgacctggaagggcgatgagaagaccagaaaccctacacctgctgtgacaccacagcctaggggcgccgagtttcacatgtggaattaccacagccacgtgttctctgtgggcgacaccttctccctggccatgcacctgcagtataagatccatgaggccccatttgatctgctgctggagtggctgtacgtgccaatcgatccaacctgccagcctatgcggctgtatagcacctgtctgtaccaccctaacgctccccagtgcctgagccacatgaatagcggatgtacctttacctctcctcacctggcccagagagtggcctctaccgtgtaccaaaactgtgagcatgccgacaattacaccgcctactgtctgggcatcagccacatggagccctctttcggcctgatcctgcatgatggaggcaccaccctgaaattcgtggataccccagagagcctgagcggcctgtatgtgtttgtggtgtacttcaatggccacgtggaggccgtggcctatacagtggtgagcacagtggatcactttgtgaacgccatcgaggaaagaggctttcctcctacagccggacagccacctgccaccaccaagcctaaggagattaccccagtgaatccaggaacaagcccactgctgaggtggccatggtatatctggctgggattcatcgccggcctgattgccatcgtgatggtgaccatcatgctgtgctgcatgaccagctgttgttcttgcctgaagggctgttgcagctgcggcagctgctgcaag

SEQ ID NO: 35 - RNA, 1743 nt, synthetic construct
  source 1..1743: mol_type = other RNA
atgggcaccgtgaataagcccgtggtgggcgtgctgatgggctttggcattatcaccggcaccctgaggatcaccaatccagtgagagcctctgtgctgaggtacgacgacttccacatcgacgaggacaagctggacaccaatagcgtgtacgagccctactaccacagcgaccatgccgagtcaagctgggtgaatagaggagagagcagcagaaaggcctacgaccacaacagcccatacatctggcccaggaacgactacgatggcttcctggagaatgctcacgagcatcacggcgtgtacaaccagggaagaggcatcgattctggagaaaggctgatgcagcctacccagatgtctgcccaggaggatctgggcgatgatacaggaatccatgtgatccctaccctgaacggcgacgacaggcacaagatcgtgaacgtggaccagaggcagtacggcgatgtgtttaagggcgacctgaatcctaagcctcagggacagaggctgatcgaggtgagcgtggaagagaatcaccctttcaccctgagagcccctatccagaggatctacggcgtgaggtatacagagacatggagctttctgccttctctgacctgcaccggagatgccgcccctgccattcagcacatctgcctgaaacacaccacctgctttcaggacgtggtggtggacgttgattgtgccgagaacaccaaggaggatcagctggccgaaatcagctataggttccagggcaagaaggaggccgatcagccctggattgtggtgaataccagcacactgtttgacgagctggagctggaccctcctgagatcgagcctggagtgctgaaggtgctgaggaccgagaagcagtacctgggagtgtacatttggaacatgaggggctctgacggcacaagcacatatgccaccttcctggtgacctggaagggcgatgagaagaccagaaaccctacacctgctgtgacaccacagcctaggggcgccgagtttcacatgtggaattaccacagccacgtgttctctgtgggcgacaccttctccctggccatgcacctgcagtataaaatccacgaggccccatttgatctgctgctggagtggctgtatgtgcccatcgatccaacctgccagcctatgcggctgtatagcacctgtctgtaccaccctaacgctccccagtgcctgagccacatgaatagcggatgtacctttacctctcctcacctggcccagagagtggcctctaccgtgtaccaaaactgtgagcatgccgacaactataccgcctactgtctgggcatcagccacatggagccctctttcggcctgatcctgcatgatggaggcaccaccctgaaattcgtggataccccagagagcctgagcggcctgtatgtgtttgtggtgtacttcaatggccacgtggaggccgtggcctatacagtggtgagcacagtggatcactttgtgaacgccatcgaggaaagaggctttcctcctacagccggacagccacctgccaccaccaagcctaaggagattaccccagtgaatccaggaacaagcccactgctgaggtggccatggtatatctggctgggattcatcgccggcctgattgccatcgtgatggtgaccatcatgctgtgctgcatgaccagctgttgttcttgcctgaagggctgttgcagctgtggcagctgctgcaag

SEQ ID NO: 36 - RNA, 1743 nt, synthetic construct
  source 1..1743: mol_type = other RNA
atgggcaccgtgaataagcccgtggtgggcgtgctgatgggatttggcattatcaccggcaccctgaggatcaccaatcctgtgagagcctctgtgctgaggtacgacgacttccacatcgacgaggacaagctggacaccaatagcgtgtacgagccctactaccactctgaccacgccgagtcaagctgggtgaatagaggagagagcagcaggaaggcctacgaccacaactctccttacatctggcccaggaacgactatgacggcttcctggagaatgctcacgagcatcacggcgtgtacaaccagggacggggaatcgattctggagaaaggctgatgcagcctacccagatgtctgcccaggaagacctgggcgatgatacaggaatccatgtgatccctaccctgaacggcgacgacaggcacaagatcgtgaacgtggaccagaggcagtacggcgatgtgtttaagggcgatctgaatcccaaacctcagggccagaggctgatcgaggtgagcgtggaggagaatcaccctttcacactgagagcccctatccagaggatctacggcgtgaggtacacagaaacatggagctttctgccttctctgacctgcaccggagatgccgcccctgccattcagcacatctgcctgaaacacaccacctgctttcaggacgtggtggtggacgttgattgtgccgagaacaccaaggaggatcagctggccgaaatcagctataggttccagggcaagaaggaggccgatcagccctggattgtggtgaataccagcacactgtttgacgagctggagctggaccctcctgagatcgagcctggagtgctgaaggtgctgaggaccgagaagcagtacctgggagtgtacatttggaacatgaggggctctgacggcacaagcacatatgccaccttcctggtgacctggaagggcgatgagaagaccagaaaccctacacctgctgtgacaccacagcctaggggcgccgagtttcacatgtggaattaccatagccacgtgttctctgtgggcgacaccttctccctggccatgcacctgcagtataagatccacgaggccccattcgatctgctgctggagtggctgtatgtgccaatcgatccaacctgccagcctatgcggctgtattctacctgtctgtaccatcccaacgccccccagtgcctgagccacatgaatagcggatgtacctttacctctcctcacctggcccagagagtggcctctaccgtgtaccaaaactgtgagcatgccgacaactataccgcctattgcctgggcatcagccacatggaacccagcttcggcctgatcctgcatgatggaggcaccaccctgaaattcgtggataccccagagagcctgagcggcctgtacgtgtttgtggtgtatttcaatggccacgtggaggccgtggcctatacagtggtgagcacagtggatcactttgtgaacgccatcgaggaaagaggctttcctcctacagccggacagccacctgccaccaccaagcctaaggagattaccccagtgaacccaggaacaagcccactgctgaggtggccatggtatatctggctgggattcatcgccggcctgattgccatcgtgatggtgaccatcatgctgtgctgtatgaccagctgttgttcttgcctgaagggctgttgtagctgtggcagctgctgcaag

SEQ ID NO: 37 - protein, 24 aa, synthetic construct
YPYDVPDYAGSSGVSGWRLFKKIS

SEQ ID NO: 38 - protein, 647 aa, synthetic construct
MGTVNKPVVGVLMGFGIITGTLRITNPVRASVLRYDDFHIDEDKLDTNSVYEPYYHSDHAESSWVNRGESSRKAYDHNSPYIWPRNDYDGFLENAHEHHGVYNQGRGIDSGERLMQPTQMSAQEDLGDDTGIHVIPTLNGDDRHKIVNVDQRQYGDVFKGDLNPKPQGQRLIEVSVEENHPFTLRAPIQRIYGVRYTETWSFLPSLTCTGDAAPAIQHICLKHTTCFQDVVVDVDCAENTKEDQLAEISYRFQGKKEADQPWIVVNTSTLFDELELDPPEIEPGVLKVLRTEKQYLGVYIWNMRGSDGTSTYATFLVTWKGDEKTRNPTPAVTPQPRGAEFHMWNYHSHVFSVGDTFSLAMHLQYKIHEAPFDLLLEWLYVPIDPTCQPMRLYSTCLYHPNAPQCLSHMNSGCTFTSPHLAQRVASTVYQNCEHADNYTAYCLGISHMEPSFGLILHDGGTTLKFVDTPESLSGLYVFVVYFNGHVEAVAYTVVSTVDHFVNAIEERGFPPTAGQPPATTKPKEITPVNPGTSPLLRYAAWTGGLAAVVLLCLVIFLICTAKRMRVKAARVDKSPYNQSMGYAGLPVDDFEDAEAADAEEEFGNAIGGSHGGSSYTVYIDKTRYPYDVPDYAGSSGVSGWRLFKKIS

SEQ ID NO: 39 - RNA, 1869 nt, synthetic construct
  source 1..1869: mol_type = other RNA
atgggcaccgtgaacaagcctgtggtgggcgtcctgatgggatttggaatcattacaggcaccctgaggatcaccaaccccgtgagagccagcgtgctgaggtacgatgacttccacatcgacgaggacaagctggacaccaacagcgtgtacgagccctactaccacagcgatcacgctgagagctcttgggtgaatagaggcgagagcagcagaaaggcctacgaccacaatagcccttacatttggcccagaaacgactacgacggctttctggagaacgcccacgagcaccacggcgtgtacaatcagggaagaggcatcgattctggagagcgactgatgcagcctacccagatgtctgcccaggaggatctgggcgatgatacaggcattcacgtgatccctaccctgaatggcgacgacagacacaagatcgtgaatgtggaccagaggcagtacggcgatgtgttcaagggcgatctgaaccccaagccacagggacagaggctgattgaggtgtctgtggaggagaatcaccctttcaccctgagagccccaatccagaggatctacggcgtgaggtacaccgaaacatggagcttcctgccttctctgacatgtaccggcgatgccgctccagccattcagcacatctgtctgaagcacaccacctgcttccaggatgtggtggtggatgtggattgcgccgagaataccaaggaggatcagctggccgagatcagctacagattccagggcaagaaagaggccgatcagccatggatcgtggtgaacaccagcacactgtttgacgagctggagctggacccacctgagattgagccaggcgtgctgaaggtgctgagaaccgagaagcagtacctgggagtgtacatctggaacatgagaggcagcgatggcacctctacctacgccacatttctggtgacctggaagggcgatgagaaaaccaggaatcctacacctgccgtgacaccccagcctagaggcgccgagtttcacatgtggaattaccacagccacgtgttcagcgtgggcgacacattcagcctggccatgcacctgcagtacaagattcacgaagccccatttgacctgctgctggagtggctgtacgtgcctatcgatcctacatgccagccaatgaggctgtacagcacctgcctgtaccacccaaatgcccctcagtgcctgagccacatgaatagcggatgtaccttcacctctcctcacctggctcagagagtggccagcacagtgtaccagaattgtgagcacgccgataactacaccgcctactgcctgggcatttctcacatggagccatcctttggcctgatcctgcatgatggcggcaccaccctgaagtttgtggatacccccgagagcctgtctggcctgtacgtgttcgtggtgtatttcaacggccacgtggaagccgtggcctatacagtggtgtctacagtggatcactttgtgaacgccatcgaggagagaggatttccccctacagctggacagcctcctgccaccaccaaacctaaggagatcacccccgtgaatcctggcacatctccactgctgagatacgctgcctggacaggaggcctggctgctgtggtgctgctgtgtctggtgatttttctgatctgtaccgccaaaagaatgagagtgaaagccgccagagtggataagagcccctacaaccagagcatgtatggcgccggcctgcctgtggatgattttgaggatgccgaggctgctgatgccgaagaggagtttggcaatgccattggcggcagccacggcggcagcagctacaccgtgtacatcgacaagaccaga

SEQ ID NO: 40 - RNA, 1869 nt, synthetic construct
  source 1..1869: mol_type = other RNA
atgggcaccgtgaataagcctgtggtgggcgtcctgatgggatttggaatcatcacaggcaccctgaggatcaccaaccccgtgagagccagcgtgctgaggtacgatgacttccacatcgacgaggacaagctggacaccaacagcgtgtacgagccctattaccatagcgatcacgccgagagctcttgggtgaatagaggcgagagcagcagaaaggcctacgaccacaacagcccttacatctggcccagaaacgactacgatggctttctggagaacgcccacgagcaccacggcgtgtacaatcagggaagaggcatcgattctggagagcgactgatgcagccaacccagatgtctgcccaggaggatctgggcgatgatacaggaatccacgtgatccctaccctgaatggcgacgacagacacaagatcgtgaatgtggaccagaggcagtacggcgacgtgtttaagggcgatctgaaccccaagccacagggacagaggctgattgaggtgtctgtggaggagaatcaccctttcaccctgagagccccaatccagaggatctacggcgtgaggtacaccgaaacatggagcttcctgccttctctgacatgtaccggcgatgccgctccagccattcagcacatctgtctgaagcacaccacctgctttcaggatgtggtggtggacgtggattgcgccgagaataccaaggaggaccagctggccgagatttcttacaggttccagggcaagaaagaggccgatcagccatggatcgtggtgaacaccagcacactgtttgacgagctggagctggacccacctgagattgagccaggcgtgctgaaggtgctgagaaccgagaagcagtacctgggagtgtacatctggaacatgagaggcagcgacggcacctctacctatgccacatttctggtgacctggaagggcgatgagaaaaccaggaatcctacacctgccgtgacaccccagcctagaggcgccgagtttcacatgtggaattaccacagccacgtgttcagcgtgggcgacacatttagcctggccatgcacctgcagtacaagatccacgaggccccattcgacctgctgttagagtggctgtatgtgcctatcgaccctacatgccagccaatgaggctgtacagcacctgtctgtaccacccaaatgcccctcagtgcctgagccacatgaacagcggatgtaccttcacctctcctcacctggctcagagagtggccagcacagtgtaccagaattgtgagcacgccgacaactacaccgcctattgcctgggcatcagccacatggagccatcttttggcttaatcctgcacgatggcggcaccaccctgaagtttgtggacacccccgaatctctgtctggcctgtacgtgttcgtggtgtatttcaacggccacgtggaagccgtggcctacacagtggtgtctacagtggatcacttcgtgaacgccatcgaagagagaggctttccccctacagctggacagcctcctgctaccacaaagcctaaggagatcacccccgtgaatcctggcacatctcccctgctgagatatgccgcttggacaggaggcctggctgctgtggtgctgctgtgtctggtgatttttctgatctgtaccgccaaaaggatgagagtgaaagccgccagagtggataagagcccctataaccagagcatgtacggcgccggcctgcctgtggatgattttgaggatgccgaggctgctgatgccgaagaggagtttggcaatgccattggcggcagccacggcggcagcagctacaccgtgtacatcgacaagaccaga

SEQ ID NO: 41 - RNA, 1869 nt, synthetic construct
  source 1..1869: mol_type = other RNA
atgggcaccgtgaataagcctgtggtgggcgtcctgatgggatttggaatcatcacaggcaccctgaggatcaccaaccccgtgagagccagcgtgctgaggtacgatgacttccacatcgacgaggacaagctggacaccaatagcgtgtacgagccctattaccatagcgaccacgccgagagctcttgggtgaacagaggcgagagcagcagaaaggcttacgatcacaacagcccttatatctggcccagaaacgactacgacggcttcctggagaacgcccacgagcaccacggcgtgtacaatcagggaagaggcatcgattctggagagcgactgatgcagccaacccagatgtctgcccaggaggatttaggcgatgacaccggaatccacgtgatccctaccctgaatggcgacgacagacacaagatcgtgaatgtggatcagaggcagtacggcgacgtgttcaagggcgacctgaacccaaagccacagggccagaggctgattgaagtgagcgtggaggagaatcacccttttaccctgagggccccaatccagaggatttatggcgtgaggtataccgagacatggagcttcctgcctagcctgacatgtaccggcgatgccgctccagccatccagcacatctgcctgaaacacaccacctgctttcaggacgtggtggtggatgttgattgcgccgagaacaccaaggaagatcagctggccgagatctcttataggttccagggcaagaaagaggccgaccagccatggatcgtggtgaataccagcacactgttcgacgagctggagctggacccacctgagattgagccaggcgtgctgaaagtgctgagaaccgagaagcagtacctgggagtgtacatctggaacatgagaggcagcgacggcacctctacctacgccacatttctggtgacctggaagggcgatgagaaaaccaggaatcccacacctgctgtgacaccccagcctagaggcgccgagtttcacatgtggaattaccacagccacgtgttcagcgtgggcgacacatttagcctggccatgcacctgcagtacaagatccacgaggccccattcgacctgctgttagagtggctgtatgtgcctatcgaccctacatgccagccaatgaggctgtacagcacctgtctgtaccacccaaatgcccctcagtgcctgagccacatgaacagcggatgtacattcacctctcctcacctggctcagagagtggccagcacagtgtaccagaattgtgagcacgccgacaactacaccgcctattgcctgggcatcagccacatggagccctctttcggcttaattctgcatgacggcggcaccacactgaagtttgtggacacccccgaatctctgtctggcctgtacgtgttcgtggtgtattttaacggccacgtggaggccgtggcctacacagtggtgtctacagtggatcacttcgtgaacgccatcgaggagagaggctttccccctacagctggacagcctcctgctaccacaaaacctaaggagatcacccccgtgaatcctggcacatctcccctgctgagatatgccgcttggacaggaggcctggctgctgtggtgctgctgtgtctggtgatttttctgatctgtaccgccaaaaggatgagagtgaaagccgccagagtggataagagcccctataatcagagcatgtacggcgccggcctgcctgtggatgatttcgaggatgccgaggctgctgatgccgaagaggagtttggcaatgccattggcggaagccacggcggcagcagctacaccgtgtacatcgacaagaccaga